European Patent Application EP 4 494 649 A1, published January 22, 2025. Title: Peptides for use in the treatment of axonal damage in diabetes. Applicant: Universitaet zu Koeln. The sequence listing filed with the application follows.

SEQUENCE LISTING (17 sequences)

SEQ ID NO: 1 - protein, 24 aa, homo sapiens
LVESCKEAFWDRCLSVINLMSSKM

SEQ ID NO: 2 - protein, 11 aa, human immunodeficieny virus
YARAARRAARR

SEQ ID NO: 3 - protein, 35 aa, synthetic construct
  REGION 1..35: note = Fusion peptide
LVESCKEAFWDRCLSVINLMSSKMYARAARRAARR

SEQ ID NO: 4 - protein, 24 aa, Homo sapiens
KEAFWDRCLSVINLMSSKMLQINA

SEQ ID NO: 5 - protein, 29 aa, Homo sapiens
ELQAVLLTCLYLSYSYMGNEISYPLKPFL

SEQ ID NO: 6 - protein, 47 aa, Homo sapiens
ELQAVLLTCLYLSYSYMGNEISYPLKPFLVESCKEAFWDRCLSVINL

SEQ ID NO: 7 - protein, 41 aa, Homo sapiens
MGNEISYPLKPFLVESCKEAFWDRCLSVINLMSSKMLQINA

SEQ ID NO: 8 - protein, 57 aa, Homo sapiens
ELQAVLLTCLYLSYSYMGNEISYPLKPFLVESCKEAFWDRCLSVINLMSSKMLQINA

SEQ ID NO: 9 - protein, 11 aa, human immunodeficiency virus
YGRKKRRQRRR

SEQ ID NO: 10 - protein, 10 aa, human immunodeficiency virus
GRKKRRQRRR

SEQ ID NO: 11 - protein, 12 aa, human immunodeficiency virus
GRKKRRQRRRPQ

SEQ ID NO: 12 - protein, 9 aa, human immunodeficiency virus
RKKRRQRRR

SEQ ID NO: 13 - protein, 35 aa, synthetic construct
  REGION 1..35: note = fusion peptide
KEAFWDRCLSVINLMSSKMLQINAYARAARRAARR

SEQ ID NO: 14 - DNA, 20 bp, synthetic construct
  misc_feature 1..20: note = primer
  source 1..20: mol_type = other DNA
taagcctttacccccctcca

SEQ ID NO: 15 - DNA, 20 bp, synthetic construct
  misc_feature 1..20: note = primer
  source 1..20: mol_type = other DNA
atccttgagccaggataccg

SEQ ID NO: 16 - DNA, 21 bp, synthetic construct
  misc_feature 1..21: note = primer
  source 1..21: mol_type = other DNA
agctgtcctcttgagattact

SEQ ID NO: 17 - DNA, 20 bp, synthetic construct
  misc_feature 1..20: note = primer
  source 1..20: mol_type = other DNA
ggaagtctcagaatgtcctc